European Patent Application EP 4 248 743 A1, published September 27, 2023. Title: Method for producing a transgenic non-human animal having a genome comprising a humanized immunoglobulin locus. Applicant: HUMAB CO., LTD. The sequence listing filed with the application follows.

SEQUENCE LISTING (56 sequences)

SEQ ID NO: 1 - DNA, 34 bp, Unknown
  Lox m2/71
taccgttcgtatatggtttcttatacgaagttat

SEQ ID NO: 2 - DNA, 34 bp, Unknown
  LoxP variant (Lox m2/66)
ataacttcgtatatggtttcttatacgaacggta

SEQ ID NO: 3 - DNA, 34 bp, Unknown
  LoxP variant (Lox 71)
taccgttcgtatagcatacattatacgaagttat

SEQ ID NO: 4 - DNA, 34 bp, Unknown
  LoxP variant (Lox 66)
ataacttcgtatagcatacattatacgaacggta

SEQ ID NO: 5 - DNA, 48 bp, Unknown
  FRT sequence
gaagttcctatactttctagagaataggaacttcggaataggaacttc

SEQ ID NO: 6 - DNA, 100 bp, Unknown
  phiC31-attP sequence
cccaggtcagaagcggttttcgggagtagtgccccaactggggtaacctttgagttctctcagttgggggcgtagggtcgccgacatgacacaaggggtt

SEQ ID NO: 7 - DNA, 70 bp, Unknown
  phiC31-attB sequence
ctcgaagccgcggtgcgggtgccagggcgtgcccttgggctccccgggcgcgtactccacctcacccatc

SEQ ID NO: 8 - DNA, 63 bp, Unknown
  PiggyBac right(3') ITR sequence
ccctagaaagataatcatattgtgacgtacgttaaagataatcatgcgtaaaattgacgcatg

SEQ ID NO: 9 - DNA, 35 bp, Unknown
  PiggyBac left(5') ITR sequence
catgcgtcaattttacgcagactatctttctaggg

SEQ ID NO: 10 - protein, 342 aa, Unknown
  Cre Recombinase
SNLLTVHQNLPALPVDATSDEVRKNLMDMFRDRQAFSEHTWKMLLSVCRSWAAWCKLNNRKWFPAEPEDVRDYLLYLQARGLAVKTIQQHLGQLNMLHRRSGLPRPSDSNAVSLVMRRIRKENVDAGERAKQALAFERTDFDQVRSLMENSDRCQDIRNLAFLGIAYNTLLRIAEIARIRVKDISRTDGGRMLIHIGRTKTLVSTAGVEKALSLGVTKLVERWISVSGVADDPNNYLFCRVRKNGVAAPSATSQLSTRALEGIFEATHRLIYGAKDDSGQRYLAWSGHSARVGAARDMARAGVSIPEIMQAGGWTNVNIVMNYIRNLDSETGAMVRLLEDGD

SEQ ID NO: 11 - protein, 594 aa, Unknown
  Piggy Bac Transposase
MGSSLDDEHILSALLQSDDELVGEDSDSEISDHVSEDDVQSDTEEAFIDEVHEVQPTSSGSEILDEQNVIEQPGSSLASNRILTLPQRTIRGKNKHCWSTSKSTRRSRVSALNIVRSQRGPTRMCRNIYDPLLCFKLFFTDEIISEIVKWTNAEISLKRRESMTGATFRDTNEDEIYAFFGILVMTAVRKDNHMSTDDLFDRSLSMVYVSVMSRDRFDFLIRCLRMDDKSIRPTLRENDVFTPVRKIWDLFIHQCIQNYTPGAHLTIDEQLLGFRGRCPFRMYIPNKPSKYGIKILMMCDSGTKYMINGMPYLGRGTQTNGVPLGEYYVKELSKPVHGSCRNITCDNWFTSIPLAKNLLQEPYKLTIVGTVRSNKREIPEVLKNSRSRPVGTSMFCFDGPLTLVSYKPKPAKMVYLLSSCDEDASINESTGKPQMVMYYNQTKGGVDTLDQMCSVMTCSRKTNRWPMALLYGMINIACINSFIIYSHNVSSKGEKVQSRKKFMRNLYMSLTSSFMRKRLEAPTLKRYLRDNISNILPNEVPGTSDDSTEEPVMKKRTYCTYCPSKIRRKANASCKKCKKVICREHNIDMCQSCF

SEQ ID NO: 12 - DNA, 34 bp, Artificial Sequence
  Primer (NeoR-EcoRI-forward)
gaattcggctgtggaatgtgtgtcagttagggtg

SEQ ID NO: 13 - DNA, 77 bp, Artificial Sequence
  Primer (NeoR-loxp-bridge)
cttatcatgtctgtataccgtcgcgccaccataacttcgtatagcatacattatacgaagttatcggtcgacgtcgg

SEQ ID NO: 14 - DNA, 20 bp, Artificial Sequence
  Primer (NeoR-SalI-reverse)
ccgacgtcgaccgataactt

SEQ ID NO: 15 - DNA, 32 bp, Artificial Sequence
  Primer (M001-SalI-forward)
acgcgtcgacaggatttggacctgagcatact

SEQ ID NO: 16 - DNA, 31 bp, Artificial Sequence
  Primer (M001-XhoI-reverse)
ccgctcgaggaggccaagagaggctaaagcc

SEQ ID NO: 17 - DNA, 31 bp, Artificial Sequence
  Primer (M002-BamHI-forward)
cgcggatcccattctcccatctccaatttat

SEQ ID NO: 18 - DNA, 29 bp, Artificial Sequence
  Primer (M002-EcoRI-reverse)
ggaattcttttgtaacccctagacagatg

SEQ ID NO: 19 - DNA, 23 bp, Artificial Sequence
  Primer (CMV-HindIII-forward)
aagcttccgccatgttgacattg

SEQ ID NO: 20 - DNA, 16 bp, Artificial Sequence
  Primer (CMV-reverse, 5'-phosphorylated)
cggccgccctatagtg

SEQ ID NO: 21 - DNA, 25 bp, Artificial Sequence
  Primer (GFP-Neo-forward, 5'-phosphorylated)
agatggagagcgacgagagcggcct

SEQ ID NO: 22 - DNA, 32 bp, Artificial Sequence
  Primer (H001-SalI-forward)
acgcgtcgactgcgtgagatcttttcttgggg

SEQ ID NO: 23 - DNA, 31 bp, Artificial Sequence
  Primer (H001-XhoI-reverse)
ccgctcgagtccacacacccaagtcattcga

SEQ ID NO: 24 - DNA, 31 bp, Artificial Sequence
  Primer (H002-BamHI-forward)
cgcggatccctgaagccaaccaagtttagga

SEQ ID NO: 25 - DNA, 31 bp, Artificial Sequence
  Primer (H002-HindIII-reverse)
cccaagcttcacatggtgaacccaaacactc

SEQ ID NO: 26 - DNA, 28 bp, Artificial Sequence
  Primer (CMV-XhoI-forward)
atcctcgaggacattgattattgactag

SEQ ID NO: 27 - DNA, 25 bp, Artificial Sequence
  Primer (CMV-KpnI-reverse)
attggtaccctcggccgccctatag

SEQ ID NO: 28 - DNA, 73 bp, Artificial Sequence
  Primer (Hygro-loxm2/71-KpnI-forward)
ataggtacctaccgttcgtatatggtttcttatacgaagttatgaattccaccatgaaaaagcctgaactcac

SEQ ID NO: 29 - DNA, 64 bp, Artificial Sequence
  Primer (Hygro-lox66-SalI-reverse)
atcgtcgactaccgttcgtataatgtatgctatacgaagttatggatcctaagatacattgatg

SEQ ID NO: 30 - DNA, 74 bp, Artificial Sequence
  Primer (Puro-deltaTK-lox71-XhoI-forward)
attctcgagataacttcgtataatgtatgctatacgaacggtaatcgatccccagcatgcctgctattgtcttc

SEQ ID NO: 31 - DNA, 76 bp, Artificial Sequence
  Primer (Puro-deltaTK-loxm2/66-HindIII-reverse)
ctcaagcttataacttcgtatatggtttcttatacgaacggtacttaagcaccatggggaccgagtacaagcccac

SEQ ID NO: 32 - DNA, 28 bp, Artificial Sequence
  Primer (Neo-HindIII-forward)
cgcaagcttgtgtgtcagttagggtgtg

SEQ ID NO: 33 - DNA, 30 bp, Artificial Sequence
  Primer (Neo-SalI-reverse)
atcgtcgactaagatacattgatgagtttg

SEQ ID NO: 34 - DNA, 21 bp, Artificial Sequence
  Primer (mIgHP-left-F2)
ttggtcctcctccttctaagc

SEQ ID NO: 35 - DNA, 20 bp, Artificial Sequence
  Primer (EF1a-R3)
gccataacccgtaaagaggc

SEQ ID NO: 36 - DNA, 21 bp, Artificial Sequence
  Primer (HygR-R1)
ccgatggctgtgtagaagtac

SEQ ID NO: 37 - DNA, 24 bp, Artificial Sequence
  Primer (mTV2-targeting Right F2)
atttcacactgcatatttcaccca

SEQ ID NO: 38 - DNA, 21 bp, Artificial Sequence
  Primer (mIgHM-left-F1)
actctgatgtctaggaccagg

SEQ ID NO: 39 - DNA, 21 bp, Artificial Sequence
  Primer (CAG-R1)
acgcggaactccatatatggg

SEQ ID NO: 40 - DNA, 21 bp, Artificial Sequence
  Primer (TK-F1)
tcctggattacgaccaatcgc

SEQ ID NO: 41 - DNA, 21 bp, Artificial Sequence
  Primer (mIgHM-right-R1)
cttcacgtcactgactgactg

SEQ ID NO: 42 - DNA, 21 bp, Artificial Sequence
  Primer (hTV2-left-F5)
ctgcagacatcaccctcattc

SEQ ID NO: 43 - DNA, 21 bp, Artificial Sequence
  Primer (hTV2-right-R4)
gtaagaagggtggagacacag

SEQ ID NO: 44 - DNA, 21 bp, Artificial Sequence
  Primer (hIgHM-left-F1)
tgtggctacaagtgcttggag

SEQ ID NO: 45 - DNA, 21 bp, Artificial Sequence
  Primer (Neo-F2)
tgtcatctcaccttgctcctg

SEQ ID NO: 46 - DNA, 21 bp, Artificial Sequence
  Primer (hIgHM-right-R1)
gtgcgatgatgacctacagtc

SEQ ID NO: 47 - DNA, 21 bp, Artificial Sequence
  Primer (mIgKP-left-F1)
ttccacagctgttgcctatcc

SEQ ID NO: 48 - DNA, 21 bp, Artificial Sequence
  Primer (mIgKP-right-R1)
caaggttcctgactaccactg

SEQ ID NO: 49 - DNA, 21 bp, Artificial Sequence
  Primer (mIgKC-left-F1)
gaagtgaagtctgccagttcc

SEQ ID NO: 50 - DNA, 21 bp, Artificial Sequence
  Primer (PuroR-F3)
tgcaagaactcttcctcacgc

SEQ ID NO: 51 - DNA, 21 bp, Artificial Sequence
  Primer (mIgKC-right-R1)
tgcactgccttcagagtgtag

SEQ ID NO: 52 - DNA, 21 bp, Artificial Sequence
  Primer (hIgKP-left-F2)
actcgtgtgaacgcgtcatac

SEQ ID NO: 53 - DNA, 21 bp, Artificial Sequence
  Primer (hIgKC-right-R2)
cctaacaacaaccacaaccac

SEQ ID NO: 54 - DNA, 21 bp, Artificial Sequence
  Primer (hIgKC-left-F2)
tctggaactgcctctgttgtg

SEQ ID NO: 55 - DNA, 21 bp, Artificial Sequence
  Primer (hIgKC-right-R2)
catagctggattatgcctgcc

SEQ ID NO: 56 - DNA, 21 bp, Artificial Sequence
  Primer (hIgKP-right-R5)
acagacagctaatgtggtggc